European Patent Application EP 4 574 973 A1, published June 25, 2025. Title: Novel promoter for constitutive expression, target protein expresssion system including same, and manufacturing method of allulose using the same. Applicant: DAESANG CORPORATION. The sequence listing filed with the application follows.

SEQUENCE LISTING (28 sequences)

SEQ ID NO: 1 - DNA, 336 bp, Corynebacterium glutamicum
  source 1..336: mol_type = genomic DNA
cagcttgcatgcctgcagaagcgcctcatcagcggtaaccatcacgggttcgggtgcgaaaaaccatgccataacaggaatgttcctttcgaaaattgaggaagccttatgcccttcaaccctacttagctgccaattattccgggcttgtgacccgctacccgataaataggtcggctgaaaaatttcgttgcaatatcaacaaaaaggcctatcattgggaggtgtcgcaccaagtacttttgcgaagcgccatctgacggattttcaaaagatgtatatgctcggtgcggaaacctacgaaaggattttttacccatgaacccgattggaatg

SEQ ID NO: 2 - DNA, 300 bp, Corynebacterium glutamicum
  source 1..300: mol_type = genomic DNA
aagcgcctcatcagcggtaaccatcacgggttcgggtgcgaaaaaccatgccataacaggaatgttcctttcgaaaattgaggaagccttatgcccttcaaccctacttagctgccaattattccgggcttgtgacccgctacccgataaataggtcggctgaaaaatttcgttgcaatatcaacaaaaaggcctatcattgggaggtgtcgcaccaagtacttttgcgaagcgccatctgacggattttcaaaagatgtatatgctcggtgcggaaacctacgaaaggattttttaccc

SEQ ID NO: 3 - DNA, 282 bp, Corynebacterium glutamicum
  source 1..282: mol_type = genomic DNA
cagcttgcatgcctgcagaacaggaatgttcctttcgaaaattgaggaagccttatgcccttcaaccctacttagctgccaattattccgggcttgtgacccgctacccgataaataggtcggctgaaaaatttcgttgcaatatcaacaaaaaggcctatcattgggaggtgtcgcaccaagtacttttgcgaagcgccatctgacggattttcaaaagatgtatatgctcggtgcggaaacctacgaaaggattttttacccatgaacccgattggaatg

SEQ ID NO: 4 - DNA, 246 bp, Corynebacterium glutamicum
  source 1..246: mol_type = genomic DNA
aacaggaatgttcctttcgaaaattgaggaagccttatgcccttcaaccctacttagctgccaattattccgggcttgtgacccgctacccgataaataggtcggctgaaaaatttcgttgcaatatcaacaaaaaggcctatcattgggaggtgtcgcaccaagtacttttgcgaagcgccatctgacggattttcaaaagatgtatatgctcggtgcggaaacctacgaaaggattttttaccc

SEQ ID NO: 5 - DNA, 236 bp, Corynebacterium glutamicum
  source 1..236: mol_type = genomic DNA
cagcttgcatgcctgcagaccctacttagctgccaattattccgggcttgtgacccgctacccgataaataggtcggctgaaaaatttcgttgcaatatcaacaaaaaggcctatcattgggaggtgtcgcaccaagtacttttgcgaagcgccatctgacggattttcaaaagatgtatatgctcggtgcggaaacctacgaaaggattttttacccatgaacccgattggaatg

SEQ ID NO: 6 - DNA, 200 bp, Corynebacterium glutamicum
  source 1..200: mol_type = genomic DNA
accctacttagctgccaattattccgggcttgtgacccgctacccgataaataggtcggctgaaaaatttcgttgcaatatcaacaaaaaggcctatcattgggaggtgtcgcaccaagtacttttgcgaagcgccatctgacggattttcaaaagatgtatatgctcggtgcggaaacctacgaaaggattttttaccc

SEQ ID NO: 7 - DNA, 176 bp, Corynebacterium glutamicum
  source 1..176: mol_type = genomic DNA
cagcttgcatgcctgcagtgaaaaatttcgttgcaatatcaacaaaaaggcctatcattgggaggtgtcgcaccaagtacttttgcgaagcgccatctgacggattttcaaaagatgtatatgctcggtgcggaaacctacgaaaggattttttacccatgaacccgattggaatg

SEQ ID NO: 8 - DNA, 140 bp, Corynebacterium glutamicum
  source 1..140: mol_type = genomic DNA
tgaaaaatttcgttgcaatatcaacaaaaaggcctatcattgggaggtgtcgcaccaagtacttttgcgaagcgccatctgacggattttcaaaagatgtatatgctcggtgcggaaacctacgaaaggattttttaccc

SEQ ID NO: 9 - DNA, 36 bp, synthetic construct
  source 1..36: mol_type = other DNA
cagcttgcatgcctgcagaagcgcctcatcagcggt

SEQ ID NO: 10 - DNA, 36 bp, synthetic construct
  source 1..36: mol_type = other DNA
cagcttgcatgcctgcagaacaggaatgttcctttc

SEQ ID NO: 11 - DNA, 36 bp, synthetic construct
  source 1..36: mol_type = other DNA
cagcttgcatgcctgcagaccctacttagctgccaa

SEQ ID NO: 12 - DNA, 36 bp, synthetic construct
  source 1..36: mol_type = other DNA
cagcttgcatgcctgcagtgaaaaatttcgttgcaa

SEQ ID NO: 13 - DNA, 36 bp, synthetic construct
  source 1..36: mol_type = other DNA
cattccaatcgggttcatgggtaaaaaatcctttcg

SEQ ID NO: 14 - protein, 294 aa, Flavonifractor plautii
MNPIGMHYGFWSHNWDEIAYIPLMEKLAWLGFDICEVASAEWGYYDDARLRELKACADHNGLGITYSIGLEAKYDLASDDPAVRENGIRHVTRILESMPKVGAAILNGVSYAGWQALPDHGITLDEKRRKEELALESMSRLMKVAEDCGVLYCCEVVNRFEQYLLNTAKEGVEFVKRLGSPNARVLLDTFHMNIEEDSMVDAILEAGPWLGHFHVGENNRRPAGSTNRLPWKDMAAALKQVNYQGAIVMEPFVLMGGTIPYDIKVWRDLSGGAGEAGLDEMAGRACRFLKELTA

SEQ ID NO: 15 - DNA, 885 bp, Flavonifractor plautii
  source 1..885: mol_type = genomic DNA
atgaacccgattggaatgcactacggcttctggagccacaactgggacgagattgcatacatacccctgatggagaagctggcctggctgggctttgacatctgcgaggtggcctccgccgagtggggctattacgacgacgccaggctgcgggagctgaaggcctgcgccgatcacaacggcctgggcatcacctattccatcggcctggaggccaaatacgacctggccagcgacgatccggcggtgcgggagaacggcatccgccatgtcacccgcatcctggagagcatgcccaaggtgggggcggccatcctcaacggcgtgtcctacgccgggtggcaggccctgcccgaccacggaatcaccctggacgagaagcgccgcaaggaggagcttgccctggagtccatgtcccggctcatgaaggtggcggaggactgcggcgtgctctactgctgcgaggtggtcaaccgcttcgagcagtacctgctcaacaccgccaaagagggcgtggagtttgtcaagcgcctgggcagtcccaacgcccgggtgctgctggataccttccacatgaacatcgaggaggacagcatggtggacgccattctggaggcgggcccctggctggggcatttccacgtgggggagaacaaccgccgccccgccggctccaccaaccgcctgccctggaaggacatggccgccgccctcaagcaggtgaactaccagggggccattgtgatggagcccttcgtgctcatggggggtaccattccctatgatatcaaggtctggcgggatctcagcggcggggccggggaggccgggctggacgagatggcgggccgggcctgccggttcctcaaggagctgaccgcgtaa

SEQ ID NO: 16 - protein, 294 aa, synthetic construct
MNPIGMHYGFWSHNWDEIAYIPLMEKLAKLGFDICEVASAEWGYYDDARLRELKACADHNGLGITYSIGLEAKYDLASDDPAVRENGIRHVTRILESMPKVGAAILNGVSYAGWQALPDHGITLDEKRRKEELALESMSRLMKVAEDCGVLYCCEVVNRFEQYLLNTAKEGVEFVKRLGSPNARVLLDTFHMNIEEDSMVDAILEAGPWLGHFHVSENNRRPAGSTNRLPWKDIAAALKQVNYQGAIVMEPFVLMGGTIPYDIKVWRDLSGGAGEAGLDEMAGRACRFLKELTA

SEQ ID NO: 17 - DNA, 885 bp, synthetic construct
  source 1..885: mol_type = other DNA
atgaacccgattggaatgcactacggcttctggagccacaactgggacgagattgcatacatacccctgatggagaagctggccaaactgggctttgacatctgcgaggtggcctccgccgagtggggctattacgacgacgccaggctgcgggagctgaaggcctgcgccgatcacaacggcctgggcatcacctattccatcggcctggaggccaaatacgacctggccagcgacgatccggcggtgcgggagaacggcatccgccatgtcacccgcatcctggagagcatgcccaaggtgggggcggccatcctcaacggcgtgtcctacgccgggtggcaggccctgcccgaccacggaatcaccctggacgagaagcgccgcaaggaggagcttgccctggagtccatgtcccggctcatgaaggtggcggaggactgcggcgtgctctactgctgcgaggtggtcaaccgcttcgagcagtacctgctcaacaccgccaaagagggcgtggagtttgtcaagcgcctgggcagtcccaacgcccgggtgctgctggataccttccacatgaacatcgaggaggacagcatggtggacgccattctggaggcgggcccctggctggggcatttccacgtgagcgagaacaaccgccgccccgccggctccaccaaccgcctgccctggaaggacattgccgccgccctcaagcaggtgaactaccagggggccattgtgatggagcccttcgtgctcatggggggtaccattccctatgatatcaaggtctggcgggatctcagcggcggggccggggaggccgggctggacgagatggcgggccgggcctgccggttcctcaaggagctgaccgcgtaa

SEQ ID NO: 18 - protein, 294 aa, synthetic construct
MNPIGMHYGFWSHNWDEIAYIPLMEKLAKLGFDICEVASAEWGYYDDARLRELKACADHNGLGITYSIGLEAKYDLSSDDPAVRENGIRHVTRILESMPKVGAAILNGVSYAGWQALPDHGITLDEKRRKEELALESMSRLMKVAEDCGVLYCCEVVNRFEQYLLNTAKEGVEFVKRLGSPNARVLLDTFHMNIEEDSMVDAILEAGPWLGHFHVSENNRRPAGSTNRLPWKDIAAALKQVNYQGAIVMEPFVLMGGTIPYDIKVWRDLSGGAGEAGLDEMAGRACRFLKELTA

SEQ ID NO: 19 - DNA, 885 bp, synthetic construct
  source 1..885: mol_type = other DNA
atgaacccgattggaatgcactacggcttctggagccacaactgggacgagattgcatacatacccctgatggagaagctggccaaactgggctttgacatctgcgaggtggcctccgccgagtggggctattacgacgacgccaggctgcgggagctgaaggcctgcgccgatcacaacggcctgggcatcacctattccatcggcctggaggccaaatacgacctgagcagcgacgatccggcggtgcgggagaacggcatccgccatgtcacccgcatcctggagagcatgcccaaggtgggggcggccatcctcaacggcgtgtcctacgccgggtggcaggccctgcccgaccacggaatcaccctggacgagaagcgccgcaaggaggagcttgccctggagtccatgtcccggctcatgaaggtggcggaggactgcggcgtgctctactgctgcgaggtggtcaaccgcttcgagcagtacctgctcaacaccgccaaagagggcgtggagtttgtcaagcgcctgggcagtcccaacgcccgggtgctgctggataccttccacatgaacatcgaggaggacagcatggtggacgccattctggaggcgggcccctggctggggcatttccacgtgagcgagaacaaccgccgccccgccggctccaccaaccgcctgccctggaaggacattgccgccgccctcaagcaggtgaactaccagggggccattgtgatggagcccttcgtgctcatggggggtaccattccctatgatatcaaggtctggcgggatctcagcggcggggccggggaggccgggctggacgagatggcgggccgggcctgccggttcctcaaggagctgaccgcgtaa

SEQ ID NO: 20 - DNA, 921 bp, synthetic construct
  source 1..921: mol_type = other DNA
cgaaaggattttttacccatgaacccgattggaatgcactacggcttctggagccacaactgggacgagattgcatacatacccctgatggagaagctggccaaactgggctttgacatctgcgaggtggcctccgccgagtggggctattacgacgacgccaggctgcgggagctgaaggcctgcgccgatcacaacggcctgggcatcacctattccatcggcctggaggccaaatacgacctgagcagcgacgatccggcggtgcgggagaacggcatccgccatgtcacccgcatcctggagagcatgcccaaggtgggggcggccatcctcaacggcgtgtcctacgccgggtggcaggccctgcccgaccacggaatcaccctggacgagaagcgccgcaaggaggagcttgccctggagtccatgtcccggctcatgaaggtggcggaggactgcggcgtgctctactgctgcgaggtggtcaaccgcttcgagcagtacctgctcaacaccgccaaagagggcgtggagtttgtcaagcgcctgggcagtcccaacgcccgggtgctgctggataccttccacatgaacatcgaggaggacagcatggtggacgccattctggaggcgggcccctggctggggcatttccacgtgagcgagaacaaccgccgccccgccggctccaccaaccgcctgccctggaaggacattgccgccgccctcaagcaggtgaactaccagggggccattgtgatggagcccttcgtgctcatggggggtaccattccctatgatatcaaggtctggcgggatctcagcggcggggccggggaggccgggctggacgagatggcgggccgggcctgccggttcctcaaggagctgaccgcgtaaggatccccgggtgggaaa

SEQ ID NO: 21 - DNA, 36 bp, synthetic construct
  source 1..36: mol_type = other DNA
cgaaaggattttttacccatgaacccgattggaatg

SEQ ID NO: 22 - DNA, 36 bp, synthetic construct
  source 1..36: mol_type = other DNA
tttcccacccggggatccttacgcggtcagctcctt

SEQ ID NO: 23 - DNA, 1185 bp, synthetic construct
  source 1..1185: mol_type = other DNA
aagcgcctcatcagcggtaaccatcacgggttcgggtgcgaaaaaccatgccataacaggaatgttcctttcgaaaattgaggaagccttatgcccttcaaccctacttagctgccaattattccgggcttgtgacccgctacccgataaataggtcggctgaaaaatttcgttgcaatatcaacaaaaaggcctatcattgggaggtgtcgcaccaagtacttttgcgaagcgccatctgacggattttcaaaagatgtatatgctcggtgcggaaacctacgaaaggattttttacccatgaacccgattggaatgcactacggcttctggagccacaactgggacgagattgcatacatacccctgatggagaagctggccaaactgggctttgacatctgcgaggtggcctccgccgagtggggctattacgacgacgccaggctgcgggagctgaaggcctgcgccgatcacaacggcctgggcatcacctattccatcggcctggaggccaaatacgacctgagcagcgacgatccggcggtgcgggagaacggcatccgccatgtcacccgcatcctggagagcatgcccaaggtgggggcggccatcctcaacggcgtgtcctacgccgggtggcaggccctgcccgaccacggaatcaccctggacgagaagcgccgcaaggaggagcttgccctggagtccatgtcccggctcatgaaggtggcggaggactgcggcgtgctctactgctgcgaggtggtcaaccgcttcgagcagtacctgctcaacaccgccaaagagggcgtggagtttgtcaagcgcctgggcagtcccaacgcccgggtgctgctggataccttccacatgaacatcgaggaggacagcatggtggacgccattctggaggcgggcccctggctggggcatttccacgtgagcgagaacaaccgccgccccgccggctccaccaaccgcctgccctggaaggacattgccgccgccctcaagcaggtgaactaccagggggccattgtgatggagcccttcgtgctcatggggggtaccattccctatgatatcaaggtctggcgggatctcagcggcggggccggggaggccgggctggacgagatggcgggccgggcctgccggttcctcaaggagctgaccgcgtaa

SEQ ID NO: 24 - DNA, 1131 bp, synthetic construct
  source 1..1131: mol_type = other DNA
aacaggaatgttcctttcgaaaattgaggaagccttatgcccttcaaccctacttagctgccaattattccgggcttgtgacccgctacccgataaataggtcggctgaaaaatttcgttgcaatatcaacaaaaaggcctatcattgggaggtgtcgcaccaagtacttttgcgaagcgccatctgacggattttcaaaagatgtatatgctcggtgcggaaacctacgaaaggattttttacccatgaacccgattggaatgcactacggcttctggagccacaactgggacgagattgcatacatacccctgatggagaagctggccaaactgggctttgacatctgcgaggtggcctccgccgagtggggctattacgacgacgccaggctgcgggagctgaaggcctgcgccgatcacaacggcctgggcatcacctattccatcggcctggaggccaaatacgacctgagcagcgacgatccggcggtgcgggagaacggcatccgccatgtcacccgcatcctggagagcatgcccaaggtgggggcggccatcctcaacggcgtgtcctacgccgggtggcaggccctgcccgaccacggaatcaccctggacgagaagcgccgcaaggaggagcttgccctggagtccatgtcccggctcatgaaggtggcggaggactgcggcgtgctctactgctgcgaggtggtcaaccgcttcgagcagtacctgctcaacaccgccaaagagggcgtggagtttgtcaagcgcctgggcagtcccaacgcccgggtgctgctggataccttccacatgaacatcgaggaggacagcatggtggacgccattctggaggcgggcccctggctggggcatttccacgtgagcgagaacaaccgccgccccgccggctccaccaaccgcctgccctggaaggacattgccgccgccctcaagcaggtgaactaccagggggccattgtgatggagcccttcgtgctcatggggggtaccattccctatgatatcaaggtctggcgggatctcagcggcggggccggggaggccgggctggacgagatggcgggccgggcctgccggttcctcaaggagctgaccgcgtaa

SEQ ID NO: 25 - DNA, 1085 bp, synthetic construct
  source 1..1085: mol_type = other DNA
accctacttagctgccaattattccgggcttgtgacccgctacccgataaataggtcggctgaaaaatttcgttgcaatatcaacaaaaaggcctatcattgggaggtgtcgcaccaagtacttttgcgaagcgccatctgacggattttcaaaagatgtatatgctcggtgcggaaacctacgaaaggattttttacccatgaacccgattggaatgcactacggcttctggagccacaactgggacgagattgcatacatacccctgatggagaagctggccaaactgggctttgacatctgcgaggtggcctccgccgagtggggctattacgacgacgccaggctgcgggagctgaaggcctgcgccgatcacaacggcctgggcatcacctattccatcggcctggaggccaaatacgacctgagcagcgacgatccggcggtgcgggagaacggcatccgccatgtcacccgcatcctggagagcatgcccaaggtgggggcggccatcctcaacggcgtgtcctacgccgggtggcaggccctgcccgaccacggaatcaccctggacgagaagcgccgcaaggaggagcttgccctggagtccatgtcccggctcatgaaggtggcggaggactgcggcgtgctctactgctgcgaggtggtcaaccgcttcgagcagtacctgctcaacaccgccaaagagggcgtggagtttgtcaagcgcctgggcagtcccaacgcccgggtgctgctggataccttccacatgaacatcgaggaggacagcatggtggacgccattctggaggcgggcccctggctggggcatttccacgtgagcgagaacaaccgccgccccgccggctccaccaaccgcctgccctggaaggacattgccgccgccctcaagcaggtgaactaccagggggccattgtgatggagcccttcgtgctcatggggggtaccattccctatgatatcaaggtctggcgggatctcagcggcggggccggggaggccgggctggacgagatggcgggccgggcctgccggttcctcaaggagctgaccgcgtaa

SEQ ID NO: 26 - DNA, 1025 bp, synthetic construct
  source 1..1025: mol_type = other DNA
tgaaaaatttcgttgcaatatcaacaaaaaggcctatcattgggaggtgtcgcaccaagtacttttgcgaagcgccatctgacggattttcaaaagatgtatatgctcggtgcggaaacctacgaaaggattttttacccatgaacccgattggaatgcactacggcttctggagccacaactgggacgagattgcatacatacccctgatggagaagctggccaaactgggctttgacatctgcgaggtggcctccgccgagtggggctattacgacgacgccaggctgcgggagctgaaggcctgcgccgatcacaacggcctgggcatcacctattccatcggcctggaggccaaatacgacctgagcagcgacgatccggcggtgcgggagaacggcatccgccatgtcacccgcatcctggagagcatgcccaaggtgggggcggccatcctcaacggcgtgtcctacgccgggtggcaggccctgcccgaccacggaatcaccctggacgagaagcgccgcaaggaggagcttgccctggagtccatgtcccggctcatgaaggtggcggaggactgcggcgtgctctactgctgcgaggtggtcaaccgcttcgagcagtacctgctcaacaccgccaaagagggcgtggagtttgtcaagcgcctgggcagtcccaacgcccgggtgctgctggataccttccacatgaacatcgaggaggacagcatggtggacgccattctggaggcgggcccctggctggggcatttccacgtgagcgagaacaaccgccgccccgccggctccaccaaccgcctgccctggaaggacattgccgccgccctcaagcaggtgaactaccagggggccattgtgatggagcccttcgtgctcatggggggtaccattccctatgatatcaaggtctggcgggatctcagcggcggggccggggaggccgggctggacgagatggcgggccgggcctgccggttcctcaaggagctgaccgcgtaa

SEQ ID NO: 27 - DNA, 197 bp, synthetic construct
  source 1..197: mol_type = other DNA
accctacttagctgccaattattccgggcttgtgacccgctacccgataaataggtcggctgaaaaatttcgttgcaatatcaacaaaaaggcctatcattgggaggtgtcgcaccaagtacttttgcgaagcgccatctgacggattttcaaaagatgtatatgctcggtgcggaaacctacgaaaggattttcat

SEQ ID NO: 28 - DNA, 1082 bp, synthetic construct
  source 1..1082: mol_type = other DNA
accctacttagctgccaattattccgggcttgtgacccgctacccgataaataggtcggctgaaaaatttcgttgcaatatcaacaaaaaggcctatcattgggaggtgtcgcaccaagtacttttgcgaagcgccatctgacggattttcaaaagatgtatatgctcggtgcggaaacctacgaaaggattttcatatgaacccgattggaatgcactacggcttctggagccacaactgggacgagattgcatacatacccctgatggagaagctggccaaactgggctttgacatctgcgaggtggcctccgccgagtggggctattacgacgacgccaggctgcgggagctgaaggcctgcgccgatcacaacggcctgggcatcacctattccatcggcctggaggccaaatacgacctgagcagcgacgatccggcggtgcgggagaacggcatccgccatgtcacccgcatcctggagagcatgcccaaggtgggggcggccatcctcaacggcgtgtcctacgccgggtggcaggccctgcccgaccacggaatcaccctggacgagaagcgccgcaaggaggagcttgccctggagtccatgtcccggctcatgaaggtggcggaggactgcggcgtgctctactgctgcgaggtggtcaaccgcttcgagcagtacctgctcaacaccgccaaagagggcgtggagtttgtcaagcgcctgggcagtcccaacgcccgggtgctgctggataccttccacatgaacatcgaggaggacagcatggtggacgccattctggaggcgggcccctggctggggcatttccacgtgagcgagaacaaccgccgccccgccggctccaccaaccgcctgccctggaaggacattgccgccgccctcaagcaggtgaactaccagggggccattgtgatggagcccttcgtgctcatggggggtaccattccctatgatatcaaggtctggcgggatctcagcggcggggccggggaggccgggctggacgagatggcgggccgggcctgccggttcctcaaggagctgaccgcgtaa